European Patent Application EP 4 775 595 A1, published July 15, 2026. Title: IGF-1R及TSHR结合蛋白及其医药用途. Applicant: 北京拓界生物医药科技有限公司. Application WO. The sequence listing filed with the application follows.

SEQUENCE LISTING (61 sequences)

SEQ ID NO: 1 - protein, 948 aa, synthetic construct
  source 1..948: note = hIGF-1R-ECD-avi-his
EICGPGIDIRNDYQQLKRLENCTVIEGYLHILLISKAEDYRSYRFPKLTVITEYLLLFRVAGLESLGDLFPNLTVIRGWKLFYNYALVIFEMTNLKDIGLYNLRNITRGAIRIEKNADLCYLSTVDWSLILDAVSNNYIVGNKPPKECGDLCPGTMEEKPMCEKTTINNEYNYRCWTTNRCQKMCPSTCGKRACTENNECCHPECLGSCSAPDNDTACVACRHYYYAGVCVPACPPNTYRFEGWRCVDRDFCANILSAESSDSEGFVIHDGECMQECPSGFIRNGSQSMYCIPCEGPCPKVCEEEKKTKTIDSVTSAQMLQGCTIFKGNLLINIRRGNNIASELENFMGLIEVVTGYVKIRHSHALVSLSFLKNLRLILGEEQLEGNYSFYVLDNQNLQQLWDWDHRNLTIKAGKMYFAFNPKLCVSEIYRMEEVTGTKGRQSKGDINTRNNGERASCESDVLHFTSTTTSKNRIIITWHRYRPPDYRDLISFTVYYKEAPFKNVTEYDGQDACGSNSWNMVDVDLPPNKDVEPGILLHGLKPWTQYAVYVKAVTLTMVENDHIRGAKSEILYIRTNASVPSIPLDVLSASNSSSQLIVKWNPPSLPNGNLSYYIVRWQRQPQDGYLYRHNYCSKDKIPIRKYADGTIDIEEVTENPKTEVCGGEKGPCCACPKTEAEKQAEKEEAEYRKVFENFLHNSIFVPRPERKRRDVMQVANTTMSSRSRNTTAADTYNITDPEELETEYPFFESRVDNKERTVISNLRPFTLYRIDIHSCNHEAEKLGCSASNFVFARTMPAEGADDIPGPVTWEPRPENSIFLKWPEPENPNGLILMYEIKYGSQVEDQRECVSRQEYRKYGGAKLNRLNPGNYTARIQATSLSGNGSWTDPVFFYVQAKTGYENFIHGGGGSGGGGSGLNDIFEAQKIEWHEGGGGSGGGGSHHHHHHHH

SEQ ID NO: 2 - protein, 284 aa, synthetic construct
  source 1..284: note = hTSHR-ECD-avi-his
GMGCSSPPCECHQEEDFRVTCKDIQRIPSLPPSTQTLKLIETCLRTIPSHAFSNLPNISRIYVSIDVTLQQLESHSFYNLSKVTHIEIRNTPNLTYIDPDALKELPLLKFLGIFNTGLKMFPPLTKVYSTEIFFILEITDNPYMTSIPRNAFQGLCNETLTLKLYNNGFTSVQGYAFNGTKLDAVYLNKNKYLTVIDKDAFGGVYSGPSLLDVSQTSVTALPSKGLEHLKELRARNTWTLGGGGGSGGGGSGLNDIFEAQKIEWHEGGGGSGGGGSHHHHHHHH

SEQ ID NO: 3 - protein, 521 aa, synthetic construct
  source 1..521: note = hTSHR-ECD-camel Fc-avi-his
GMGCSSPPCECHQEEDFRVTCKDIQRIPSLPPSTQTLKLIETCLRTIPSHAFSNLPNISRIYVSIDVTLQQLESHSFYNLSKVTHIEIRNTPNLTYIDPDALKELPLLKFLGIFNTGLKMFPPLTKVYSTEIFFILEITDNPYMTSIPRNAFQGLCNETLTLKLYNNGFTSVQGYAFNGTKLDAVYLNKNKYLTVIDKDAFGGVYSGPSLLDVSQTSVTALPSKGLEHLKELRARNTWTLLEISEPQPQPGCTCPKCPAPELPGGPSVFVFPPKPKDVLSISGRPEVTCVVVDVGKEDPEVNFNWYIDGVEVRTANTKPKEEQFNSTYRVVSVLTIQHQDWLTGKEFKCKVNNKALPAPIERTISKAKGQTREPQVYTLAPHREELAKDTVSVTCLVKGFYPPDINVEWQRNRQPESEGAYATTLPQLDNDGTYFLYSKLSVGKNTWQRGETFTCVVMHEALHNHYTQKSITQSSGKGGGGGSGGGGSGLNDIFEAQKIEWHEGGGGSGGGGSHHHHHHHH

SEQ ID NO: 4 - protein, 128 aa, synthetic construct
  source 1..128: note = IG05
QVQLVESGGGLVQAGGSLRLSCTASGLTFGTFGMAWFRQAPGKEREGVSAISASSGRTYYADSVKGRFTISRDNAKNTLYLQMDALKPEDTAMYYCAVRSKNGAGYGFWYEARLYGYWGQGTQVTVSS

SEQ ID NO: 5 - protein, 120 aa, synthetic construct
  source 1..120: note = IG06
QVQLVESGGGSVQAGGSLRLSCAASRYIVSTRCLGWVRQAPGNEREEIATIDTAGRPTYADSVKGRFTISKDGAKNFLYLQMNSLKPEDTAMYYCAAASSDNCRYFPSNLGQGTQVTVSS

SEQ ID NO: 6 - protein, 129 aa, synthetic construct
  source 1..129: note = CB16
EVQLVESGGGPVQAGGSLRLSCAGPGYTSSCMGWFRQAPGKERTGVAAIYIGGRGTDYADSVKGRFTISQDNAKNTLYLQMNSLKPEDTAMYYCWAGIEYDCYSGHWRDWAFSRERGFWGQGTQVTVSS

SEQ ID NO: 7 - protein, 5 aa, synthetic construct
  source 1..5: note = IG05 CDR1
TFGMA

SEQ ID NO: 8 - protein, 17 aa, synthetic construct
  source 1..17: note = IG05 CDR2
AISASSGRTYYADSVKG

SEQ ID NO: 9 - protein, 19 aa, synthetic construct
  source 1..19: note = IG05 CDR3
RSKNGAGYGFWYEARLYGY

SEQ ID NO: 10 - protein, 5 aa, synthetic construct
  source 1..5: note = IG06 CDR1
TRCLG

SEQ ID NO: 11 - protein, 16 aa, synthetic construct
  source 1..16: note = IG06 CDR2
TIDTAGRPTYADSVKG

SEQ ID NO: 12 - protein, 12 aa, synthetic construct
  source 1..12: note = IG06 CDR3
ASSDNCRYFPSN

SEQ ID NO: 13 - skipped

SEQ ID NO: 14 - protein, 17 aa, synthetic construct
  source 1..17: note = CB16 CDR2
AIYIGGRGTDYADSVKG

SEQ ID NO: 15 - protein, 22 aa, synthetic construct
  source 1..22: note = CB16 CDR3
GIEYDCYSGHWRDWAFSRERGF

SEQ ID NO: 16 - protein, 231 aa, Homo sapiens
  source 1..231: note; note (original language) = 人IgG1 Fc区
EPKSSDKTHTCPPCPAPELLGGPSVFLFPPKPKDTLMISRTPEVTCVVVDVSHEDPEVKFNWYVDGVEVHNAKTKPREEQYNSTYRVVSVLTVLHQDWLNGKEYKCKVSNKALPAPIEKTISKAKGQPREPQVYTLPPSRDELTKNQVSLTCLVKGFYPSDIAVEWESNGQPENNYKTTPPVLDSDGSFFLYSKLTVDKSRWQQGNVFSCSVMHEALHNHYTQKSLSLSPG

SEQ ID NO: 17 - protein, 359 aa, synthetic construct
  source 1..359: note = IG05-IgG1
QVQLVESGGGLVQAGGSLRLSCTASGLTFGTFGMAWFRQAPGKEREGVSAISASSGRTYYADSVKGRFTISRDNAKNTLYLQMDALKPEDTAMYYCAVRSKNGAGYGFWYEARLYGYWGQGTQVTVSSEPKSSDKTHTCPPCPAPELLGGPSVFLFPPKPKDTLMISRTPEVTCVVVDVSHEDPEVKFNWYVDGVEVHNAKTKPREEQYNSTYRVVSVLTVLHQDWLNGKEYKCKVSNKALPAPIEKTISKAKGQPREPQVYTLPPSRDELTKNQVSLTCLVKGFYPSDIAVEWESNGQPENNYKTTPPVLDSDGSFFLYSKLTVDKSRWQQGNVFSCSVMHEALHNHYTQKSLSLSPG

SEQ ID NO: 18 - protein, 351 aa, synthetic construct
  source 1..351: note = IG06-IgG1
QVQLVESGGGSVQAGGSLRLSCAASRYIVSTRCLGWVRQAPGNEREEIATIDTAGRPTYADSVKGRFTISKDGAKNFLYLQMNSLKPEDTAMYYCAAASSDNCRYFPSNLGQGTQVTVSSEPKSSDKTHTCPPCPAPELLGGPSVFLFPPKPKDTLMISRTPEVTCVVVDVSHEDPEVKFNWYVDGVEVHNAKTKPREEQYNSTYRVVSVLTVLHQDWLNGKEYKCKVSNKALPAPIEKTISKAKGQPREPQVYTLPPSRDELTKNQVSLTCLVKGFYPSDIAVEWESNGQPENNYKTTPPVLDSDGSFFLYSKLTVDKSRWQQGNVFSCSVMHEALHNHYTQKSLSLSPG

SEQ ID NO: 19 - protein, 360 aa, synthetic construct
  source 1..360: note = CB16-IgG1
EVQLVESGGGPVQAGGSLRLSCAGPGYTSSCMGWFRQAPGKERTGVAAIYIGGRGTDYADSVKGRFTISQDNAKNTLYLQMNSLKPEDTAMYYCWAGIEYDCYSGHWRDWAFSRERGFWGQGTQVTVSSEPKSSDKTHTCPPCPAPELLGGPSVFLFPPKPKDTLMISRTPEVTCVVVDVSHEDPEVKFNWYVDGVEVHNAKTKPREEQYNSTYRVVSVLTVLHQDWLNGKEYKCKVSNKALPAPIEKTISKAKGQPREPQVYTLPPSRDELTKNQVSLTCLVKGFYPSDIAVEWESNGQPENNYKTTPPVLDSDGSFFLYSKLTVDKSRWQQGNVFSCSVMHEALHNHYTQKSLSLSPG

SEQ ID NO: 20 - protein, 128 aa, synthetic construct
  source 1..128: note = IG05-hu1
EVQLVESGGGLVQPGGSLRLSCTASGLTFGTFGMAWFRQAPGKEREGVSAISASSGRTYYADSVKGRFTISRDNSKNTLYLQMNSLRAEDTAVYYCAVRSKNGAGYGFWYEARLYGYWGQGTLVTVSS

SEQ ID NO: 21 - protein, 128 aa, synthetic construct
  source 1..128: note = IG05-hu2
EVQLVESGGGLVQPGGSLRLSCTASGLTFGTFGMAWFRQAPGKEREGVSAISASSGRTYYADSVKGRFTISRDNAKNTLYLQMNSLRAEDTAVYYCAVRSKNGAGYGFWYEARLYGYWGQGTLVTVSS

SEQ ID NO: 22 - protein, 128 aa, synthetic construct
  source 1..128: note = IG05-hu3
EVQLVESGGGLVQPGGSLRLSCTASGLTFGTFGMAWFRQAPGKEREGVSAISASSGRTYYADSVKGRFTISRDNSKNTLYLQMDALRAEDTAVYYCAVRSKNGAGYGFWYEARLYGYWGQGTLVTVSS

SEQ ID NO: 23 - protein, 128 aa, synthetic construct
  source 1..128: note = IG05-hu4
EVQLVESGGGLVQPGGSLRLSCAASGLTFGTFGMAWFRQAPGKEREGVSAISASSGRTYYADSVKGRFTISRDNSKNTLYLQMNSLRAEDTAVYYCAVRSKNGAGYGFWYEARLYGYWGQGTLVTVSS

SEQ ID NO: 24 - protein, 128 aa, synthetic construct
  source 1..128: note = IG05-hu5
EVQLVESGGGLVQPGGSLRLSCAASGFTFGTFGMAWFRQAPGKEREGVSAISASSGRTYYADSVKGRFTISRDNSKNTLYLQMNSLRAEDTAVYYCAVRSKNGAGYGFWYEARLYGYWGQGTLVTVSS

SEQ ID NO: 25 - protein, 120 aa, synthetic construct
  source 1..120: note = IG06-hu1
EVQLVESGGGLVQPGGSLRLSCAASRYIVSTRCLGWVRQAPGKEREEVSTIDTAGRPTYADSVKGRFTISRDNSKNTLYLQMNSLRAEDTAVYYCAAASSDNCRYFPSNWGQGTLVTVSS

SEQ ID NO: 26 - protein, 120 aa, synthetic construct
  source 1..120: note = IG06-hu2
EVQLVESGGGLVQPGGSLRLSCAASRYIVSTRCLGWVRQAPGKEREEVSTIDTAGRPTYADSVKGRFTISRDNSKNFLYLQMNSLRAEDTAVYYCAAASSDNCRYFPSNWGQGTLVTVSS

SEQ ID NO: 27 - protein, 120 aa, synthetic construct
  source 1..120: note = IG06-hu3
EVQLVESGGGLVQPGGSLRLSCAASRYIVSTRCLGWVRQAPGKEREEVSTIDTAGRPTYADSVKGRFTISRDGAKNFLYLQMNSLRAEDTAVYYCAAASSDNCRYFPSNWGQGTLVTVSS

SEQ ID NO: 28 - protein, 120 aa, synthetic construct
  source 1..120: note = IG06-hu4
EVQLVESGGGLVQPGGSLRLSCAASRYIVSTRCLGWVRQAPGKEREEVSTIDTAGRPTYADSVKGRFTISRDGAKNFLYLQMNSLRAEDTAVYYCAAASSDNCRYFPSNLGQGTLVTVSS

SEQ ID NO: 29 - protein, 120 aa, synthetic construct
  source 1..120: note = IG06-hu5
EVQLVESGGGLVQPGGSLRLSCAASRYIVSTRCLGWVRQAPGKEREEIATIDTAGRPTYADSVKGRFTISRDGAKNFLYLQMNSLRAEDTAVYYCAAASSDNCRYFPSNLGQGTLVTVSS

SEQ ID NO: 30 - protein, 120 aa, synthetic construct
  source 1..120: note = IG06-hu6
EVQLVESGGGLVQPGGSLRLSCAASRYIVSTRCLGWVRQAPGNEREEVSTIDTAGRPTYADSVKGRFTISRDNSKNTLYLQMNSLRAEDTAVYYCAAASSDNCRYFPSNLGQGTLVTVSS

SEQ ID NO: 31 - protein, 129 aa, synthetic construct
  source 1..129: note = CB16-hu1
EVQLLESGGGLVQPGGSLRLSCAGPGYTSSCMGWFRQAPGKEREGVSAIYIGGRGTDYADSVKGRFTISQDNSKNTLYLQMNSLRAEDTAVYYCWAGIEYDCYSGHWRDWAFSRERGFWGQGTLVTVSS

SEQ ID NO: 32 - protein, 129 aa, synthetic construct
  source 1..129: note = CB16-hu2
EVQLLESGGGLVQPGGSLRLSCAGPGYTSSCMGWFRQAPGKERTGVAAIYIGGRGTDYADSVKGRFTISQDNAKNTLYLQMNSLRAEDTAVYYCWAGIEYDCYSGHWRDWAFSRERGFWGQGTLVTVSS

SEQ ID NO: 33 - protein, 129 aa, synthetic construct
  source 1..129: note = CB16-hu3
EVQLLESGGGLVQPGGSLRLSCAGPGYTSSCMGWFRQAPGKERTGVSAIYIGGRGTDYADSVKGRFTISQDNSKNTLYLQMNSLRAEDTAVYYCWAGIEYDCYSGHWRDWAFSRERGFWGQGTLVTVSS

SEQ ID NO: 34 - protein, 128 aa, synthetic construct
  source 1..128: note = IG05-hu5-1
EVQLVESGGGLVQPGGSLRLSCAASGFTFGTFGMAWFRQAPGKEREGVSAISASSGRTYYADSVKGRFTISRDNSKNTLYLQMNSLRAEDTAVYYCAVRSKQGAGYGFWYEGRLYGYWGQGTLVTVSS

SEQ ID NO: 35 - protein, 19 aa, synthetic construct
  source 1..19: note = IG05 CDR3
  VARIANT 4: note; note (original language) = X为N或Q
  VARIANT 14: note; note (original language) = X为A或G
RSKXGAGYGFWYEXRLYGY

SEQ ID NO: 36 - protein, 19 aa, synthetic construct
  source 1..19: note = IG05 CDR3
RSKQGAGYGFWYEGRLYGY

SEQ ID NO: 37 - protein, 359 aa, synthetic construct
  source 1..359: note = IG05-hu5-1-IgG1
EVQLVESGGGLVQPGGSLRLSCAASGFTFGTFGMAWFRQAPGKEREGVSAISASSGRTYYADSVKGRFTISRDNSKNTLYLQMNSLRAEDTAVYYCAVRSKQGAGYGFWYEGRLYGYWGQGTLVTVSSEPKSSDKTHTCPPCPAPELLGGPSVFLFPPKPKDTLMISRTPEVTCVVVDVSHEDPEVKFNWYVDGVEVHNAKTKPREEQYNSTYRVVSVLTVLHQDWLNGKEYKCKVSNKALPAPIEKTISKAKGQPREPQVYTLPPSRDELTKNQVSLTCLVKGFYPSDIAVEWESNGQPENNYKTTPPVLDSDGSFFLYSKLTVDKSRWQQGNVFSCSVMHEALHNHYTQKSLSLSPG

SEQ ID NO: 38 - protein, 360 aa, synthetic construct
  source 1..360: note = CB16-hu3-IgG1
EVQLLESGGGLVQPGGSLRLSCAGPGYTSSCMGWFRQAPGKERTGVSAIYIGGRGTDYADSVKGRFTISQDNSKNTLYLQMNSLRAEDTAVYYCWAGIEYDCYSGHWRDWAFSRERGFWGQGTLVTVSSEPKSSDKTHTCPPCPAPELLGGPSVFLFPPKPKDTLMISRTPEVTCVVVDVSHEDPEVKFNWYVDGVEVHNAKTKPREEQYNSTYRVVSVLTVLHQDWLNGKEYKCKVSNKALPAPIEKTISKAKGQPREPQVYTLPPSRDELTKNQVSLTCLVKGFYPSDIAVEWESNGQPENNYKTTPPVLDSDGSFFLYSKLTVDKSRWQQGNVFSCSVMHEALHNHYTQKSLSLSPG

SEQ ID NO: 39 - protein, 447 aa, synthetic construct
  source 1..447: note; note (original language) = Tepezza抗体重链
QVELVESGGGVVQPGRSQRLSCAASGFTFSSYGMHWVRQAPGKGLEWVAIIWFDGSSTYYADSVRGRFTISRDNSKNTLYLQMNSLRAEDTAVYFCARELGRRYFDLWGRGTLVSVSSASTKGPSVFPLAPSSKSTSGGTAALGCLVKDYFPEPVTVSWNSGALTSGVHTFPAVLQSSGLYSLSSVVTVPSSSLGTQTYICNVNHKPSNTKVDKKVEPKSCDKTHTCPPCPAPELLGGPSVFLFPPKPKDTLMISRTPEVTCVVVDVSHEDPEVKFNWYVDGVEVHNAKTKPREEQYNSTYRVVSVLTVLHQDWLNGKEYKCKVSNKALPAPIEKTISKAKGQPREPQVYTLPPSRDELTKNQVSLTCLVKGFYPSDIAVEWESNGQPENNYKTTPPVLDSDGSFFLYSKLTVDKSRWQQGNVFSCSVMHEALHNHYTQKSLSLSPG

SEQ ID NO: 40 - protein, 215 aa, synthetic construct
  source 1..215: note; note (original language) = Tepezza抗体轻链
EIVLTQSPATLSLSPGERATLSCRASQSVSSYLAWYQQKPGQAPRLLIYDASKRATGIPARFSGSGSGTDFTLTISSLEPEDFAVYYCQQRSKWPPWTFGQGTKVESKRTVAAPSVFIFPPSDEQLKSGTASVVCLLNNFYPREAKVQWKVDNALQSGNSQESVTEQDSKDSTYSLSSTLTLSKADYEKHKVYACEVTHQGLSSPVTKSFNRGEC

SEQ ID NO: 41 - protein, 453 aa, synthetic construct
  source 1..453: note; note (original language) = VRDN-001抗体重链
QVQLVQSGAEVVKPGASVKLSCKASGYTFTSYWMHWVKQRPGQGLEWIGEINPSNGRTNYNQKFQGKATLTVDKSSSTAYMQLSSLTSEDSAVYYFARGRPDYYGSSKWYFDVWGQGTTVTVSSASTKGPSVFPLAPSSKSTSGGTAALGCLVKDYFPEPVTVSWNSGALTSGVHTFPAVLQSSGLYSLSSVVTVPSSSLGTQTYICNVNHKPSNTKVDKKVEPKSCDKTHTCPPCPAPELLGGPSVFLFPPKPKDTLMISRTPEVTCVVVDVSHEDPEVKFNWYVDGVEVHNAKTKPREEQYNSTYRVVSVLTVLHQDWLNGKEYKCKVSNKALPAPIEKTISKAKGQPREPQVYTLPPSRDELTKNQVSLTCLVKGFYPSDIAVEWESNGQPENNYKTTPPVLDSDGSFFLYSKLTVDKSRWQQGNVFSCSVMHEALHNHYTQKSLSLSPG

SEQ ID NO: 42 - protein, 219 aa, synthetic construct
  source 1..219: note; note (original language) = VRDN-001抗体轻链
DVVMTQTPLSLPVSLGDPASISCRSSQSIVHSNVNTYLEWYLQKPGQSPRLLIYKVSNRFSGVPDRFSGSGAGTDFTLRISRVEAEDLGIYYCFQGSHVPPTFGGGTKLEIKRTVAAPSVFIFPPSDEQLKSGTASVVCLLNNFYPREAKVQWKVDNALQSGNSQESVTEQDSKDSTYSLSSTLTLSKADYEKHKVYACEVTHQGLSSPVTKSFNRGEC

SEQ ID NO: 43 - protein, 448 aa, synthetic construct
  source 1..448: note; note (original language) = PHP1003抗体重链
QVQLQESGPGLVKPSGTLSLTCAVSGGSISSSNWWSWVRQPPGKGLEWIGEIYHSGSTNYNPSLKSRVTISVDKSKNQFSLKLSSVTAADTAVYYCARWTGRTDAFDIWGQGTMVTVSSASTKGPSVFPLAPSSKSTSGGTAALGCLVKDYFPEPVTVSWNSGALTSGVHTFPAVLQSSGLYSLSSVVTVPSSSLGTQTYICNVNHKPSNTKVDKKVEPKSCDKTHTCPPCPAPEAAGGPSVFLFPPKPKDTLMISRTPEVTCVVVDVSHEDPEVKFNWYVDGVEVHNAKTKPREEQYNSTYRVVSVLTVLHQDWLNGKEYKCKVSNKALPAPIEKTISKAKGQPREPQVYTLPPSRDELTKNQVSLTCLVKGFYPSDIAVEWESNGQPENNYKTTPPVLDSDGSFFLYSKLTVDKSRWQQGNVFSCSVMHEALHNHYTQKSLSLSPG

SEQ ID NO: 44 - protein, 219 aa, synthetic construct
  source 1..219: note; note (original language) = PHP1003抗体轻链
DVVMTQSPLSLPVTPGEPASISCRSSQSLLHSNGYNYLDWYLQKPGQSPQLLIYLGSNRASGVPDRFSGSGSGTDFTLKISRVEAEDVGVYYCMQGTHWPLTFGQGTKVEIKRTVAAPSVFIFPPSDEQLKSGTASVVCLLNNFYPREAKVQWKVDNALQSGNSQESVTEQDSKDSTYSLSSTLTLSKADYEKHKVYACEVTHQGLSSPVTKSFNRGEC

SEQ ID NO: 45 - protein, 448 aa, synthetic construct
  source 1..448: note; note (original language) = K1-70抗体重链
EVQLVQSGAEVKKPGQSLKISCKASGYSLTDNWIGWVRQKPGKGLEWMGIIYPGDSDTRYSPSFQGQVTISADKSINTAYLQWSSLKASDTAIYYCVGLDWNYNPLRYWGPGTLVTVSSASTKGPSVFPLAPSSKSTSGGTAALGCLVKDYFPEPVTVSWNSGALTSGVHTFPAVLQSSGLYSLSSVVTVPSSSLGTQTYICNVNHKPSNTKVDKKVEPKSCDKTHTCPPCPAPELLGGPSVFLFPPKPKDTLMISRTPEVTCVVVDVSHEDPEVKFNWYVDGVEVHNAKTKPREEQYNSTYRVVSVLTVLHQDWLNGKEYKCKVSNKALPAPIEKTISKAKGQPREPQVYTLPPSRDELTKNQVSLTCLVKGFYPSDIAVEWESNGQPENNYKTTPPVLDSDGSFFLYSKLTVDKSRWQQGNVFSCSVMHEALHNHYTQKSLSLSPG

SEQ ID NO: 46 - protein, 216 aa, synthetic construct
  source 1..216: note; note (original language) = K1-70抗体轻链
QSVLTQPPSVSAAPGQKVTISCSGSSSDIGSNYVSWYQQFPGTAPKLLIYDNNKRPSAIPDRFSGSKSGTSATLGITGLQTGDEADYYCGTWDSRLGIAVFGGGTQLTVLGQPKAAPSVTLFPPSSEELQANKATLVCLVSDFYPGAVTVAWKADGSPVKVGVETTKPSKQSNNKYAASSYLSLTPEQWKSHRSYSCRVTHEGSTVEKTVAPTECS

SEQ ID NO: 47 - protein, 450 aa, synthetic construct
  source 1..450: note; note (original language) = M22抗体重链
QVQLVQSGAEVKKPGESLKISCRGSGYRFTSYWINWVRQLPGKGLEWMGRIDPTDSYTNYSPSFKGHVTVSADKSINTAYLQWSSLKASDTGMYYCARLEPGYSSTWSVNWGQGTLVTVSSASTKGPSVFPLAPSSKSTSGGTAALGCLVKDYFPEPVTVSWNSGALTSGVHTFPAVLQSSGLYSLSSVVTVPSSSLGTQTYICNVNHKPSNTKVDKKVEPKSCDKTHTCPPCPAPELLGGPSVFLFPPKPKDTLMISRTPEVTCVVVDVSHEDPEVKFNWYVDGVEVHNAKTKPREEQYNSTYRVVSVLTVLHQDWLNGKEYKCKVSNKALPAPIEKTISKAKGQPREPQVYTLPPSRDELTKNQVSLTCLVKGFYPSDIAVEWESNGQPENNYKTTPPVLDSDGSFFLYSKLTVDKSRWQQGNVFSCSVMHEALHNHYTQKSLSLSPG

SEQ ID NO: 48 - protein, 216 aa, synthetic construct
  source 1..216: note; note (original language) = M22抗体轻链
LTVLTQPPSVSGAPRQRVTISCSGNSSNIGNNAVNWYQQLPGKAPKLLIYYDDQLPSGVSDRFSGSRSGTSASLAIRGLQSEDEADYYCTSWDDSLDSQLFGGGTRLTVLGQPKAAPSVTLFPPSSEELQANKATLVCLISDFYPGAVTVAWKADSSPVKAGVETTTPSKQSNNKYAASSYLSLTPEQWKSHKSYSCQVTHEGSTVEKTVAPTECS

SEQ ID NO: 49 - protein, 503 aa, synthetic construct
  source 1..503: note = 0031-0024
EVQLVESGGGLVQPGGSLRLSCAASGFTFGTFGMAWFRQAPGKEREGVSAISASSGRTYYADSVKGRFTISRDNSKNTLYLQMNSLRAEDTAVYYCAVRSKQGAGYGFWYEGRLYGYWGQGTLVTVSSEPKSSDKTHTCPPCPAPELLGGPSVFLFPPKPKDTLMISRTPEVTCVVVDVSHEDPEVKFNWYVDGVEVHNAKTKPREEQYNSTYRVVSVLTVLHQDWLNGKEYKCKVSNKALPAPIEKTISKAKGQPREPQVYTLPPSRDELTKNQVSLTCLVKGFYPSDIAVEWESNGQPENNYKTTPPVLDSDGSFFLYSKLTVDKSRWQQGNVFSCSVMHEALHNHYTQKSLSLSPGGGGGSGGGGSGGGGSEVQLLESGGGLVQPGGSLRLSCAGPGYTSSCMGWFRQAPGKERTGVSAIYIGGRGTDYADSVKGRFTISQDNSKNTLYLQMNSLRAEDTAVYYCWAGIEYDCYSGHWRDWAFSRERGFWGQGTLVTVSS

SEQ ID NO: 50 - protein, 495 aa, synthetic construct
  source 1..495: note = 0031-0053
QVQLVESGGGSVQAGGSLRLSCAASRYIVSTRCLGWVRQAPGNEREEIATIDTAGRPTYADSVKGRFTISKDGAKNFLYLQMNSLKPEDTAMYYCAAASSDNCRYFPSNLGQGTQVTVSSEPKSSDKTHTCPPCPAPELLGGPSVFLFPPKPKDTLMISRTPEVTCVVVDVSHEDPEVKFNWYVDGVEVHNAKTKPREEQYNSTYRVVSVLTVLHQDWLNGKEYKCKVSNKALPAPIEKTISKAKGQPREPQVYTLPPSRDELTKNQVSLTCLVKGFYPSDIAVEWESNGQPENNYKTTPPVLDSDGSFFLYSKLTVDKSRWQQGNVFSCSVMHEALHNHYTQKSLSLSPGGGGGQGGGGQGGGGQEVQLLESGGGLVQPGGSLRLSCAGPGYTSSCMGWFRQAPGKERTGVSAIYIGGRGTDYADSVKGRFTISQDNSKNTLYLQMNSLRAEDTAVYYCWAGIEYDCYSGHWRDWAFSRERGFWGQGTLVTVSS

SEQ ID NO: 51 - protein, 503 aa, synthetic construct
  source 1..503: note = 0031-0060
EVQLLESGGGLVQPGGSLRLSCAGPGYTSSCMGWFRQAPGKERTGVSAIYIGGRGTDYADSVKGRFTISQDNSKNTLYLQMNSLRAEDTAVYYCWAGIEYDCYSGHWRDWAFSRERGFWGQGTLVTVSSEPKSSDKTHTCPPCPAPELLGGPSVFLFPPKPKDTLMISRTPEVTCVVVDVSHEDPEVKFNWYVDGVEVHNAKTKPREEQYNSTYRVVSVLTVLHQDWLNGKEYKCKVSNKALPAPIEKTISKAKGQPREPQVYTLPPSRDELTKNQVSLTCLVKGFYPSDIAVEWESNGQPENNYKTTPPVLDSDGSFFLYSKLTVDKSRWQQGNVFSCSVMHEALHNHYTQKSLSLSPGGGGGSGGGGSGGGGSEVQLVESGGGLVQPGGSLRLSCAASGFTFGTFGMAWFRQAPGKEREGVSAISASSGRTYYADSVKGRFTISRDNSKNTLYLQMNSLRAEDTAVYYCAVRSKQGAGYGFWYEGRLYGYWGQGTLVTVSS

SEQ ID NO: 52 - protein, 495 aa, synthetic construct
  source 1..495: note = 0031-0070
EVQLLESGGGLVQPGGSLRLSCAGPGYTSSCMGWFRQAPGKERTGVSAIYIGGRGTDYADSVKGRFTISQDNSKNTLYLQMNSLRAEDTAVYYCWAGIEYDCYSGHWRDWAFSRERGFWGQGTLVTVSSEPKSSDKTHTCPPCPAPELLGGPSVFLFPPKPKDTLMISRTPEVTCVVVDVSHEDPEVKFNWYVDGVEVHNAKTKPREEQYNSTYRVVSVLTVLHQDWLNGKEYKCKVSNKALPAPIEKTISKAKGQPREPQVYTLPPSRDELTKNQVSLTCLVKGFYPSDIAVEWESNGQPENNYKTTPPVLDSDGSFFLYSKLTVDKSRWQQGNVFSCSVMHEALHNHYTQKSLSLSPGGGGGQGGGGQGGGGQQVQLVESGGGSVQAGGSLRLSCAASRYIVSTRCLGWVRQAPGNEREEIATIDTAGRPTYADSVKGRFTISKDGAKNFLYLQMNSLKPEDTAMYYCAAASSDNCRYFPSNLGQGTQVTVSS

SEQ ID NO: 53 - protein, 5 aa, synthetic construct
  source 1..5: note; note (original language) = 连接子
GGGGS

SEQ ID NO: 54 - protein, 10 aa, synthetic construct
  source 1..10: note; note (original language) = 连接子
GGGGSGGGGS

SEQ ID NO: 55 - protein, 15 aa, synthetic construct
  source 1..15: note; note (original language) = 连接子
GGGGSGGGGSGGGGS

SEQ ID NO: 56 - protein, 20 aa, synthetic construct
  source 1..20: note; note (original language) = 连接子
GGGGSGGGGSGGGGSGGGGS

SEQ ID NO: 57 - protein, 25 aa, synthetic construct
  source 1..25: note; note (original language) = 连接子
GGGGSGGGGSGGGGSGGGGSGGGGS

SEQ ID NO: 58 - protein, 4 aa, synthetic construct
  source 1..4: note; note (original language) = 连接子
ASGS

SEQ ID NO: 59 - protein, 5 aa, synthetic construct
  source 1..5: note; note (original language) = 连接子；序列重复1-20的整数次
GGNGT

SEQ ID NO: 60 - protein, 5 aa, synthetic construct
  source 1..5: note; note (original language) = 连接子；序列重复1-20的整数次
YGNGT

SEQ ID NO: 61 - protein, 5 aa, synthetic construct
  source 1..5: note; note (original language) = 连接子；序列重复1-20的整数次
EPKSS